European Patent Application EP 4 212 550 A1, published July 19, 2023. Title: Bispecific Antibody Binding to Human Interleukin-4 receptor alpha subunit and Interleukin-5 receptor alpha subunit and Uses Thereof. Applicant: Ajou University Industry-Academic Cooperation Foundation. The sequence listing filed with the application follows.

SEQUENCE LISTING (70 sequences)

SEQ ID NO: 1 - protein, 5 aa, Artificial Sequence
  Synthetic CDR1 Sequence
RHAMA

SEQ ID NO: 2 - protein, 17 aa, Artificial Sequence
  Synthetic CDR2 Sequence
AITSSGRSIYYADSVKG

SEQ ID NO: 3 - protein, 17 aa, Artificial Sequence
  Synthetic CDR2 Sequence
AITASGRSIYYADSVKG

SEQ ID NO: 4 - protein, 17 aa, Artificial Sequence
  Synthetic CDR2 Sequence
AITASGRGIYYGDSVKG

SEQ ID NO: 5 - protein, 17 aa, Artificial Sequence
  Synthetic CDR2 Sequence
AITMSGRSIYYADSVKG

SEQ ID NO: 6 - protein, 17 aa, Artificial Sequence
  Synthetic CDR2 Sequence
AITMSGRGIYYADSVKG

SEQ ID NO: 7 - protein, 17 aa, Artificial Sequence
  Synthetic CDR2 Sequence
AITASGMSIYYADFAKG

SEQ ID NO: 8 - protein, 7 aa, Artificial Sequence
  Synthetic CDR3 Sequence
VHRAFDY

SEQ ID NO: 9 - protein, 116 aa, Artificial Sequence
  Synthetic VH Sequence
EVQLLESGGGLVQPGGSLRLSCAASGFTFSRHAMAWVRQAPGKGLEWVSAITSSGRSIYYADSVKGRFTISRDNSKNTLYLQMNSLRAEDTAVYYCARVHRAFDYWGQGTLVTVSS

SEQ ID NO: 10 - protein, 116 aa, Artificial Sequence
  Synthetic VH Sequence
EVQLLESGGGLVQPGGSLRLSCAASGFTFSRHAMAWVRQAPGKGLEWVSAITASGRSIYYADSVKGRFTISRDNSKNTLYLQMNSLRAEDTAVYYCARVHRAFDYWGQGTLVTVSS

SEQ ID NO: 11 - protein, 116 aa, Artificial Sequence
  Synthetic VH Sequence
EVQLLESGGGLVQPGGSLRLSCAASGFTFSRHAMAWVRQAPGKGLEWVSAITASGRSIYYGDSVKGRFTISRDNSKNTLYLQMNSLRAEDTAVYYCARVHRAFDYWGQGTLVTVSS

SEQ ID NO: 12 - protein, 116 aa, Artificial Sequence
  Synthetic VH Sequence
EVQLLESGGGLVQPGGSLRLSCAASGFTFSRHAMAWVRQAPGKGLEWVSAITMSGRSIYYADSVKGRFTISRDNSKNTLYLQMNSLRAEDTAVYYCARVHRAFDYWGQGTLVTVSS

SEQ ID NO: 13 - protein, 13 aa, Artificial Sequence
  Synthetic CDR1 Sequence
SGSPLFPDSGSFN

SEQ ID NO: 14 - protein, 7 aa, Artificial Sequence
  Synthetic CDR2 Sequence
ADSHRPS

SEQ ID NO: 15 - protein, 11 aa, Artificial Sequence
  Synthetic CDR3 Sequence
GTWDYSLSGYV

SEQ ID NO: 16 - protein, 11 aa, Artificial Sequence
  Synthetic CDR3 Sequence
GTWDYSLNRYV

SEQ ID NO: 17 - protein, 11 aa, Artificial Sequence
  Synthetic CDR3 Sequence
GTWDYSLSAYV

SEQ ID NO: 18 - protein, 11 aa, Artificial Sequence
  Synthetic CDR3 Sequence
GTWDYSLNSYV

SEQ ID NO: 19 - protein, 11 aa, Artificial Sequence
  Synthetic CDR3 Sequence
GTWDYSLSSYV

SEQ ID NO: 20 - protein, 11 aa, Artificial Sequence
  Synthetic CDR3 Sequence
GSWDYSLSRYV

SEQ ID NO: 21 - protein, 111 aa, Artificial Sequence
  Synthetic VL Sequence
QSVLTQPPSASGTPGQRVTISCSGSPLFPDSGSFNWYQQLPGTAPKLLIYADSHRPSGVPDRFSGSKSGTSASLAISGLRSEDEADYYCGTWDYSLSGYVLGGGTKLTVLG

SEQ ID NO: 22 - protein, 111 aa, Artificial Sequence
  Synthetic VL Sequence
QSVLTQPPSASGTPGQRVTISCSGSPLFPDSGSFNWYQQLPGTAPKLLIYADSHRPSGVPDRFSGSKSGTSASLAISGLRSEDEADYYCGTWDYSLNRYVLGGGTKLTVLG

SEQ ID NO: 23 - protein, 111 aa, Artificial Sequence
  Synthetic VL Sequence
QSVLTQPPSASGTPGQRVTISCSGSPLFPDSGSFNWYQQLPGTAPKLLIYADSHRPSGVPDRFSGSKSGTSASLAISGLRSEDEADYYCGTWDYSLSAYVLGGGTKLTVLG

SEQ ID NO: 24 - protein, 111 aa, Artificial Sequence
  Synthetic VL Sequence
QSVLTQPPSASGTPGQRVTISCSGSPLFPDSGSFNWYQQLPGTAPKLLIYADSHRPSGVPDRFSGSKSGTSASLAISGLRSEDEADYYCGTWDYSLNSYVLGGGTKLTVLG

SEQ ID NO: 25 - protein, 111 aa, Artificial Sequence
  Synthetic VL Sequence
QSVLTQPPSASGTPGQRVTISCSGSPLFPDSGSFNWYQQLPGTAPKLLIYADSHRPSGVPDRFSGSKSGTSASLAISGLRSEDEADYYCGTWDYSLSSYVLGGGTKLTVLG

SEQ ID NO: 26 - protein, 111 aa, Artificial Sequence
  Synthetic VL Sequence
QSVLTQPPSASGTPGQRVTISCSGSPLFPDSGSFNWYQQLPGTAPKLLIYADSHRPSGVPDRFSGSKSGTSASLAISGLRSEDEADYYCGTWDYSLSRYVLGGGTKLTVLG

SEQ ID NO: 27 - protein, 5 aa, Artificial Sequence
  Synthetic CDR1 Sequence
SYWIN

SEQ ID NO: 28 - protein, 17 aa, Artificial Sequence
  Synthetic CDR2 Sequence
HIYPNKNENYYNHKFKD

SEQ ID NO: 29 - protein, 13 aa, Artificial Sequence
  Synthetic CDR3 Sequence
DYYGRSYYYAMDY

SEQ ID NO: 30 - protein, 13 aa, Artificial Sequence
  Synthetic CDR3 Sequence
EFYGRQYYQAMDY

SEQ ID NO: 31 - protein, 13 aa, Artificial Sequence
  Synthetic CDR3 Sequence
EYYGRSYYAAMDY

SEQ ID NO: 32 - protein, 13 aa, Artificial Sequence
  Synthetic CDR3 Sequence
EHYGRPYYNAMDY

SEQ ID NO: 33 - protein, 13 aa, Artificial Sequence
  Synthetic CDR3 Sequence
EYYGRTYYSAMDY

SEQ ID NO: 34 - protein, 13 aa, Artificial Sequence
  Synthetic CDR3 Sequence
EFYGRSRYSAMDY

SEQ ID NO: 35 - protein, 13 aa, Artificial Sequence
  Synthetic CDR3 Sequence
EYYGRSYYNAMDY

SEQ ID NO: 36 - protein, 122 aa, Artificial Sequence
  Synthetic VH Sequence
QVQLVQSGAEVKKPGSSVKVSCKASGYTFTSYWINWVRQAPGQGLEWIGHIYPNKNENYYNHKFKDKATLTVDKSTNTAYMELSSLRSEDTAVYYCTRDYYGRSYYYAMDYWGQGTTLTVSS

SEQ ID NO: 37 - protein, 122 aa, Artificial Sequence
  Synthetic VH Sequence
QVQLVQSGAEVKKPGSSVKVSCKASGYTFTSYWINWVRQAPGQGLEWIGHIYPNKNENYYNHKFKDKATLTVDKSTNTAYMELSSLRSEDTAVYYCTREFYGRQYYQAMDYWGQGTTLTVSS

SEQ ID NO: 38 - protein, 122 aa, Artificial Sequence
  Synthetic VH Sequence
QVQLVQSGAEVKKPGSSVKVSCKASGYTFTSYWINWVRQAPGQGLEWIGHIYPNKNENYYNHKFKDKATLTVDKSTNTAYMELSSLRSEDTAVYYCTREYYGRSYYAAMDYWGQGTTLTVSS

SEQ ID NO: 39 - protein, 122 aa, Artificial Sequence
  Synthetic VH Sequence
QVQLVQSGAEVKKPGSSVKVSCKASGYTFTSYWINWVRQAPGQGLEWIGHIYPNKNENYYNHKFKDKATLTVDKSTNTAYMELSSLRSEDTAVYYCTREHYGRPYYNAMDYWGQGTTLTVSS

SEQ ID NO: 40 - protein, 122 aa, Artificial Sequence
  Synthetic VH Sequence
QVQLVQSGAEVKKPGSSVKVSCKASGYTFTSYWINWVRQAPGQGLEWIGHIYPNKNENYYNHKFKDKATLTVDKSTNTAYMELSSLRSEDTAVYYCTREYYGRTYYSAMDYWGQGTTLTVSS

SEQ ID NO: 41 - protein, 122 aa, Artificial Sequence
  Synthetic VH Sequence
QVQLVQSGAEVKKPGSSVKVSCKASGYTFTSYWINWVRQAPGQGLEWIGHIYPNKNENYYNHKFKDKATLTVDKSTNTAYMELSSLRSEDTAVYYCTREFYGRSRYSAMDYWGQGTTLTVSS

SEQ ID NO: 42 - protein, 122 aa, Artificial Sequence
  Synthetic VH Sequence
QVQLVQSGAEVKKPGSSVKVSCKASGYTFTSYWINWVRQAPGQGLEWIGHIYPNKNENYYNHKFKDKATLTVDKSTNTAYMELSSLRSEDTAVYYCTREYYGRSYYNAMDYWGQGTTLTVSS

SEQ ID NO: 43 - protein, 27 aa, Artificial Sequence
  Synthetic CDR1 Sequence
KASQNVGTAVAWASTRHTQQFGRYPYT

SEQ ID NO: 44 - protein, 7 aa, Artificial Sequence
  Synthetic CDR2 Sequence
WASTRHT

SEQ ID NO: 45 - protein, 9 aa, Artificial Sequence
  Synthetic CDR3 Sequence
QQFGRYPYT

SEQ ID NO: 46 - protein, 107 aa, Artificial Sequence
  Synthetic VL Sequence
DIQMTQSPSTLSASVGDRVTITCKASQNVGTAVAWYQQKPGKAPKLLIYWASTRHTGVPDRFSGSGSGTDFTLTISSLQPDDFATYYCQQFGRYPYTFGSGTKVEVK

SEQ ID NO: 47 - protein, 107 aa, Artificial Sequence [sequence omitted]

SEQ ID NO: 48 - protein, 59 aa, Artificial Sequence
  Synthetic Linker Sequence
GSSGSGSGSTGTSSSGTGTSAGTTGTSASTSGSGSGGGGGSGGGGSAGGTATAGASSGS

SEQ ID NO: 49 - protein, 98 aa, Artificial Sequence
  CH1
ASTKGPSVFPLAPSSKSTSGGTAALGCLVKDYFPEPVTVSWNSGALTSGVHTFPAVLQSSGLYSLSSVVTVPSSSLGTQTYICNVNHKPSNTKVDKKV

SEQ ID NO: 50 - protein, 15 aa, Artificial Sequence
  Hinge
EPKSCDKTHTCPPCP

SEQ ID NO: 51 - protein, 110 aa, Artificial Sequence
  CH2
APELLGGPSVFLFPPKPKDTLMISRTPEVTCVVVDVSHEDPEVKFNWYVDGVEVHNAKTKPREEQYNSTYRVVSVLTVLHQDWLNGKEYKCKVSNKALPAPIEKTISKAK

SEQ ID NO: 52 - protein, 107 aa, Artificial Sequence
  CH3A
GQPREPQVYTLPPSRDELTENQVSLTCLVKGFYPSDIAVEWESNGQPENNYKTTPPVLDSDGSFFLYSWLTVDKSRWQQGNVFSCSVMHEALHNHYTQKSLSLSPGK

SEQ ID NO: 53 - protein, 107 aa, Artificial Sequence
  CH3B
GQPREPRVYTLPPSRDELTKNQVSLTCLVKGFYPSDIAVEWESNGQPENNYKTTPPVLVSDGSFTLYSKLTVDKSRWQQGNVFSCSVMHEALHNHYTQKSLSLSPGK

SEQ ID NO: 54 - protein, 107 aa, Artificial Sequence
  CL_V133E
RTVAAPSVFIFPPSDEQLKSGTASVECLLNNFYPREAKVQWKVDNALQSGNSQESVTEQDSKDSTYSLSSTLTLSKADYEKHKVYACEVTHQGLSSPVTKSFNRGEC

SEQ ID NO: 55 - protein, 107 aa, Artificial Sequence
  CL_V133K
RTVAAPSVFIFPPSDEQLKSGTASVKCLLNNFYPREAKVQWKVDNALQSGNSQESVTEQDSKDSTYSLSSTLTLSKADYEKHKVYACEVTHQGLSSPVTKSFNRGEC

SEQ ID NO: 56 - protein, 107 aa, Artificial Sequence
  CH3
GQPREPQVYTLPPSRDELTKNQVSLTCLVKGFYPSDIAVEWESNGQPENNYKTTPPVLDSDGSFFLYSKLTVDKSRWQQGNVFSCSVMHEALHNHYTQKSLSLSPGK

SEQ ID NO: 57 - protein, 16 aa, Artificial Sequence
  Linker
LGGGGSGGGGSGGGGS

SEQ ID NO: 58 - protein, 122 aa, Artificial Sequence
  anti-IL-5Ralpha VH G44C
QVQLVQSGAEVKKPGSSVKVSCKASGYTFTSYWINWVRQAPGQCLEWIGHIYPNKNENYYNHKFKDKATLTVDKSTNTAYMELSSLRSEDTAVYYCTRDYYGRSYYYAMDYWGQGTTLTVSS

SEQ ID NO: 59 - protein, 20 aa, Artificial Sequence
  Linker
GGGGSGGGGSGGGGSGGGGS

SEQ ID NO: 60 - protein, 107 aa, Artificial Sequence
  anti-IL-5Ralpha VL S100C
DIQMTQSPSTLSASVGDRVTITCKASQNVGTAVAWYQQKPGKAPKLLIYWASTRHTGVPDRFSGCGSGTDFTLTISSLQPDDFATYYCQQFGRYPYTFGSGTKVEVK

SEQ ID NO: 61 - protein, 116 aa, Artificial Sequence
  anti-IL-4Ralpha VH G100C
EVQLLESGGGLVQPGGSLRLSCAASGFTFSRHAMAWVRQAPGKCLEWVSAITSSGRSIYYADSVKGRFTISRDNSKNTLYLQMNSLRAEDTAVYYCARVHRAFDYWGQGTLVTVSS

SEQ ID NO: 62 - protein, 111 aa, Artificial Sequence
  anti-IL-4Ralpha VL G44C
QSVLTQPPSASGTPGQRVTISCSGSPLFPDSGSFNWYQQLPGTAPKLLIYADSHRPSGVPDRFSGSKSGTSASLAISGLRSEDEADYYCGTWDYSLSGYVLGCGTKLTVLG

SEQ ID NO: 63 - protein, 12 aa, Artificial Sequence
  VL Long linker
TVAAPSVFIFPP

SEQ ID NO: 64 - protein, 13 aa, Artificial Sequence
  VH Long linker
ASTKGPSVFPLAP

SEQ ID NO: 65 - protein, 207 aa, Artificial Sequence
  IL-4Ralpha
MKVLQEPTCVSDYMSISTCEWKMNGPTNCSTELRLLYQLVFLLSEAHTCIPENNGGAGCVCHLLMDDVVSADNYTLDLWAGQQLLWKGSFKPSEHVKPRAPGNLTVHTNVSDTLLLTWSNPYPPDNYLYNHLTYAVNIWSENDPADFRIYNVTYLEPSLRIAASTLKSGISYRARVRAWAQCYNTTWSEWSPSTKWHNSYREPFEQH

SEQ ID NO: 66 - protein, 322 aa, Artificial Sequence
  IL-5Ralpha
DLLPDEKISLLPPVNFTIKVTGLAQVLLQWKPNPDQEQRNVNLEYQVKINAPKEDDYETRITESKCVTILHKGFSASVRTILQNDHSLLASSWASAELHAPPGSPGTSIVNLTCTTNTTEDNYSRLRSYQVSLHCTWLVGTDAPEDTQYFLYYRYGSWTEECQEYSKDTLGRNIACWFPRTFILSKGRDWLAVLVNGSSKHSAIRPFDQLFALHAIDQINPPLNVTAEIEGTRLSIQWEKPVSAFPIHCFDYEVKIHNTRNGYLQIEKLMTNAFISIIDDLSKYDVQVRAAVSSMCREAGLWSEWSQPIYVGNDEHKPLREW

SEQ ID NO: 67 - protein, 116 aa, Artificial Sequence
  Synthetic VH Sequence
EVQLLESGGGLVQPGGSLRLSCAASGFTFSRHAMAWVRQAPGKGLEWVSAITMSGRGIYYADSVKGRFTISRDNSKNTLYLQMNSLRAEDTAVYYCARVHRAFDYWGQGTLVTVSS

SEQ ID NO: 68 - protein, 116 aa, Artificial Sequence
  Synthetic VH Sequence
EVQLLESGGGLVQPGGSLRLSCAASGFTFSRHAMAWVRQAPGKGLEWVSAITASGMSIYYADFAKGRFTISRDNSKNTLYLQMNSLRAEDTAVYYCARVHRAFDYWGQGTLVTVSS

SEQ ID NO: 69 - protein, 5 aa, Artificial Sequence
  Linker
TVAAP

SEQ ID NO: 70 - protein, 6 aa, Artificial Sequence
  Linker
ASTKGP